European Patent Specification EP 3 892 631 B1, published December 13, 2023. Title: Fusion protein for use in the treatment of HvG disease. Applicant: Medizinische Hochschule Hannover Technische Universität Braunschweig. The sequence listing filed with the application follows.

SEQUENCE LISTING (25 sequences)

SEQ ID NO: 1 - protein, 251 aa, Artificial Sequence
  CHAIN 1..123: variable heavy chain
  scFv (KAZ15-C1)
  CHAIN 124..141: linker
  CHAIN 142..251: variable light chain
EVQLVQSGAEVKKPGSSVKVSCKASGGTFSSYAISWVRQAPGQGLEWMGGIIPIFGTANYAQKFQGRVTITADESTSTAYMELSSLRSEDTAVYYCARGGYDSRGSYYYMDVWGKGTTVTVSSGSASAPKLEEGEFSEARVQSVLTQPPSTSGTPGQRVTISCSGSSSNIGGNAVNWYQHFPGTAPTLLIYSNNQRPSGVPERFSGSKSGTSASLTVSGLQAEDEADYYCTAWDDSLRGYLFGTGTKVTVL

SEQ ID NO: 2 - protein, 249 aa, Artificial Sequence
  CHAIN 1..123: variable heavy chain
  scFv (KAZ15-F3)
  CHAIN 124..141: linker
  CHAIN 142..249: variable light chain
QVQLVESGGGVVQPGRSLRLSCAASGFTFSSYAMHWVRQAPGKGLEWVAVISYDGSNKYYADSVKGRFTISRDNSKNTLYLQMNSLRAEDTAVYYCARDREELLALFGGMDVWGQGTTVTVSSGSASAPKLEEGEFSEARVQPVLTQPSSVSVAPGQTARITCGGNNIGSKSVHWYQQKPGQAPVLVVYDDSDRPSGIPERFSGSNSGNTATLTISRVEARDEADYYCHVWDAKTNHQVFGGGTRLTVQ

SEQ ID NO: 3 - protein, 251 aa, Artificial Sequence
  CHAIN 1..123: variable heavy chain
  scFv (SH1319-A5)
  CHAIN 124..141: linker
  CHAIN 142..251: variable light chain
EVQLVQSGAEVKKPGSSVKVSCKASGGTFSSYAISWVRQAPGQGLEWMGGIIPIFGTANYAQKFQGRVTITADKSTSTAYMELSSLRSEDTAVYYCARPQSRWLQSGDAFDIWGQGTMVTVSSGSASAPKLEEGEFSEARVQPVLTQPRSVSGSPGQSVTISCTGTSSDVGGYNRVSWYQQTPGTAPKLMIYEVSNRPSGVSNRFSGSKSGNTASLTISGLQAEDEADYYCSSYTSSSTVVFGGGTKLTVL

SEQ ID NO: 4 - protein, 246 aa, Artificial Sequence
  CHAIN 1..119: variable heavy chain
  scFv (SH1313-B8)
  CHAIN 120..137: linker
  CHAIN 138..246: variable light chain
QVQLQQSGAEVKKPGASVKVSCKASGYTFTSYAMHWVRQAPGQRLEWMGRINAGNGNTKYSQKFQGRVTITRDTSASTAYMELSSLRSEDTAVYYCARDLTGTLLFDYWGQGTLVTVSSGSASAPKLEEGEFSEARVQSVLTQPPSASGTPGQRVTISCSGSSSNIGSNGVKWYQQLPGTAPKLVIYRDYQRPSGVPDRFSGSKSGTSASLAISGLQSEDEAKYYCAAWDDSLNVVFGGGTQLTVL

SEQ ID NO: 5 - protein, 251 aa, Artificial Sequence
  CHAIN 1..123: variable heavy chain
  scFv (SH1319-B11)
  CHAIN 124..141: linker
  CHAIN 142..251: variable light chain
QVQLVQSGAEVKKPGSSVKVSCKASGGTFSSYAISWVRQAPGQGLEWMGGIIPIFGTANYAQKFQGRATITADESTSTAYMELSSLRSEDTAVYYCARRAERWLHLSGAFDIWGQGTMVTVSSGSASAPKLEEGEFSEARVQPVLTQSSSASGTPGQRVAISCSGSSSNVGSNTVNWYQQSPGTAPKLLISSNHQRPSGVPDRFSGSKFGTSASLAISGLQSEDEADYYCGAWDDSLNGYVFGSGTKVTVL

SEQ ID NO: 6 - protein, 244 aa, Artificial Sequence
  CHAIN 1..116: variable heavy chain
  scFv (SH1319-C5)
  CHAIN 117..134: linker
  CHAIN 135..244: variable light chain
QVQLVQSGGGLVQPGGSLRLSCAASGFTFSSYAMSWVRQAPGKGLEWVSAISGSGGSTYYADSVKGRFTMSRDNAKNSLYLQMNSLRVEDSAVYYCATGHYGDYVWGQGALVTVSSGSASAPKLEEGEFSEARVQAGLTQPPSASGTPGQRVTISCSGSSSNIGSNTVNWYQQLPGTAPKLLIYSNNQRPSGVPDRFSGSKSGTSASLAISGLQSEDEADYYCAAWDDSLNGPVFGGGTKLTVL

SEQ ID NO: 7 - protein, 246 aa, Artificial Sequence
  CHAIN 1..118: variable heavy chain
  scFv (SH1319-D4)
  CHAIN 119..136: linker
  CHAIN 137..246: variable light chain
QVQLQQSGAEVKKPGASVKVSCKASGYTFTSYAMHWVRQAPGQRLEWMGWINAGNGNTKYSQKFQGRVTITRDTSASTAYMELSSLRSEDTAVYYCARVSSGGAFDIWGQGTVVTVSSGSASAPKLEEGEFSEARVQSALTQPASVSGSPGQSITISCTGTGSDVGGYKYVSWYQHHPGKAPRLIIYDVNYWPSGVSHRFSGSKSGNTASLTISGLQSEDEADYYCSSYRTGDTWVFGGGTKLTVL

SEQ ID NO: 8 - protein, 248 aa, Artificial Sequence
  CHAIN 1..123: variable heavy chain
  scFv (SH1319-D8)
  CHAIN 124..141: linker
  CHAIN 142..248: variable light chain
QVQLVQSGAEVKKPGSSVKVSCKASGGTFSSYGFSWVRQAPGQGLEWMGEIIPMFGTANYAQKLQGRVTITAETSTSTVYMELSSLRSEDTATYYCARVPRSSSGYNYGMDVWGQGTTVTVSSGSASAPKLEEGEFSEARVDIQMTQSPSSLSASVGDRVTITCRASQGISNYLAWYQQKPGKVPKLLIYAASTLQSGVPSRFSGSGSGTDFTLTISSLQPEDVATYYCQKYNSAPRTFGQGTKVEIK

SEQ ID NO: 9 - protein, 250 aa, Artificial Sequence
  CHAIN 1..122: variable heavy chain
  scFv (SH1319-E4)
  CHAIN 123..140: linker
  CHAIN 141..250: variable light chain
QVQLQQSGPGLLKPSQTLSLTCAVSGDSVSTNSGAWSWIRQSPSRGLEWLGRTYYRSKWSTDYALSLQSRVTIKSDRSKNQFSLQLDSVTPEDTAIYYCARENWNSGGFDYWGQGTLVTVPSGSASAPKLEEGEFSEARVQPVLTQSSSASGSPGQSVTISCTGTSSDVGGYNYVSWYQQHPGKAPKLMIYEVSKRPSGVPDRFSGSKSGSTASLTVSGLQAEDEAEYYCSSYAGSNNYVFGTGTKVTVL

SEQ ID NO: 10 - protein, 249 aa, Artificial Sequence
  CHAIN 1..122: variable heavy chain
  scFv (SH1319-E12)
  CHAIN 123..140: linker
  CHAIN 141..249: variable light chain
EVQLVESGAEVKKPGSSVKVSCKASGGTFSSYAISWVRQAPGQGLEWMGGIIPIFGTANYAQKFQGRVTITADKSTSTAYMELSSLRSEDTAVYYCARAASRWEPGDAFDIWGQGTMVTVSSGSASAPKLEEGEFSEARVQPVLTQSSSVSVAPGKTARVTCGGDNIGGKSVHWYQQRAGQAPVLVISHDTDRPSGIPERFSGSKSGTSASLAISGLRSEDEADYYCAVWDASLGGSWLFGGGTKLTVL

SEQ ID NO: 11 - protein, 252 aa, Artificial Sequence
  CHAIN 1..122: variable heavy chain
  scFv (SH1319-F6)
  CHAIN 123..141: linker
  CHAIN 142..252: variable light chain
QVQLVQSGAEVKKPGASVKVSCKTSGYTFTSYDISWVRQAPGQGLEWMGWISAYNGNTNYAQKLQGRVTMTTDTSTSTAYMELRRLRSDDTAVYYCARGGRWLRSASSFDYWGQGTLVTVSSGSASAPKLEEGEFSEARVQAGLTQPPSVSGAPGQRVTISCTGSSSNIGAAYDVHWYQQLPGAAPKLLIFGDSNRPSGVPDRFSGSKSDTSASLAITGLQAEDEADYYCQSFDSSLSGSRVFGGGTKLTVL

SEQ ID NO: 12 - protein, 251 aa, Artificial Sequence
  CHAIN 1..123: variable heavy chain
  scFv (SH1319-G3)
  CHAIN 124..141: linker
  CHAIN 142..251: variable light chain
EVQLVESGGGLVKPGGSLRLSCAASGFTFSDHYMSWVRQAPGKGLEWVSYITSGGSSIYYADSVKGRFTISRDNAKNSLYLQMNSLRAEDTAVYYCARGLDSSAYQGRAFDIWGQGTMVTVSSGSASAPKLEEGEFSEARVLPVLTQPPSASGTPGQRVTISCSGSSSNIGSNPVHWYQQLPGTAPKLLVYRNNQRPSGVPDRFSGSKSGTSASLAISGLRSEDEADYYCAAWDVSLSGVVFGGGTKLTVL

SEQ ID NO: 13 - protein, 81 aa, Artificial Sequence
  CD8 hinge domain and transmembran domain
FVPVFLPAKPTTTPAPRPPTPAPTIASQPLSLRPEASRPAAGGAVHTRGLDFADIYIWAPLAGTCGVLLLSLVITLYCNHR

SEQ ID NO: 14 - protein, 42 aa, Artificial Sequence
  CD28 signalling domain
WVRSKRSRLLHSDYMNMTPRRPGPTRKHYQPYAPPRDFAAYR

SEQ ID NO: 15 - protein, 113 aa, Artificial Sequence
  CD3zeta signalling domain
RVKFSRSADAPAYQQGQNQLYNELNLGRREEYDVLDKRRGRDPEMGGKPRRKNPQEGLYNELQKDKMAEAYSEIGMKGERRRGKGHDGLYQGLSTATKDTYDALHMQALPPRS

SEQ ID NO: 16 - protein, 306 aa, Artificial Sequence
  scFv (C5)
IKEEKLTMKYLLPTAAAGLLLLAAQPAMAQVQLQESGGGVIQPGRSLRLSCAASGFTFSGHGFHWVRQAPGKGLEWVAVIWYDGSKTFYADSVKGRFTISRDNSRNTVFLQMNSLRAEDTAVYYCARDLSYYAMDVRGQGTTVTVSSGSASAPKLEEGEFSEARVQTVVTQEPSLTVSPGGTVTLTCASSTGAVTSGYYPNWFQQKPGQAPRALIYSTSNKHSWTPARFSGSLLGGKAALTLSGVRPEDEAEYYCLLYYGGARVFGGGTKLTVLGQPKAAPSVTLFPPSSAAAGSEQKLISEEDLS

SEQ ID NO: 17 - protein, 315 aa, Artificial Sequence
  scFv (E4)
IKEEKLTMKYLLPTAAAGLLLLAAQPAMAQMQLVQSGAEVKKPGSSVKVSCKASGGTFSSYAISWVRQAPGQGLEWMGGIIPIFGTADYAQKFQGRVTITADESTSTAYMELSSLRSEDTAVYYCARVGPTSSSSYYYGMDVWGQGTTVTVSSGSASAPKLEEGEFSEARVQAVLTQPPSVSGAPGQRVTISCTGSSSNIGAGYDVHWYQQLPGTAPKLLIYGNSNRPSGVPDRFSGSKFGTSASLAITGLQAEDEADYYCQSFDTSLSGSKVFGGGTKLTVLGQPKAAPSVTLFPPSSAAAGSEQKLISEEDLS

SEQ ID NO: 18 - protein, 307 aa, Artificial Sequence
  scFv (F11)
MKYLLPTAAAGLLLLAAQPAMAQVQLVQSGGGVVQPGRSLRLSCAASGFTFSSYGMHWVRQAPGKGLEWVAVISYDGRNVHYADSVKGRFTISRDNSKNTLHLQMNSLRPEDSALYYCVKDLARVVITPGGMHVWGQGTTVTVSSGSAFAPKLEEGEFSEARVQAVVTQEPSLSVSPGGTVTLTCASSTGTVTGASSPNWFQQKPGQVPRPLIYGTTNKHSWTPARFSGSLLGGKAALTVSGVQPEDEAEYYCLLYSGGGQPYWMFGGGTKLTVLGQPKAAPSVTLFPPSSAAAGSEQKLISEEDLS

SEQ ID NO: 19 - protein, 310 aa, Artificial Sequence
  scFv (H7)
KEEKLTMKYLLPTAAAGLLLLAAQPAMAQVQLVQSGGGVVQPGRSLRLSCAASGFTFSSYGMHWVRQAPGKGLEWVAVISYDGSNKYYADSVKGRFTISRDNSKNTLYLQMNSLRAEDTAVYYCAKEAYNWNDGGWFDPWGQGTLVTVSSGSASAPKLEEGEFSEARVQAVLTQPPSTSGTPGQGVTISCSGSRSNIGPNYVHWYQQLPGAAPKVLIYRNYQRPSGVPDRISASKSGTSASLAISGLRSEDEAVYYCASWDDTLGAVVFGGGTKLTVLGQPKAAPSVTLFPPSSAAAGSEQKLISEEDLS

SEQ ID NO: 20 - protein, 280 aa, Artificial Sequence
  hΔFC IgG domain
MGAGATGRAMDGPRLLLLLLLGVSLGGAKEACPTGLYTHSGECCKACNLGEGVAQPCGANQTVCEPCLDSVTFSDVVSATEPCKPCTECVGLQSMSAPCVEADDAVCRCAYGYYQDETTGRCEACRVCEAGSGLVFSCQDKQNTVCEECPDGTYSDEANHVDPCLPCTVCEDTERQLRECTRWADAECEEIPGRWITRSTPPEGSDSTAPSTQEPEAPPEQDLIASTVAGVVTTVMGSSQPVVTRGTTDNLIPVYCSILAAVVVGLVAYIAFKRWNRGIL

SEQ ID NO: 21 - protein, 184 aa, Artificial Sequence
  hCD28 transmembrane domain - hCD3zeta signalling domain
DPKFWVLVVVGGVLACYSLLVTVAFIIFWVRSKRSRLLHSDYMNMTPRRPGPTRKHYQAYAAARDFAAYRSLRVKFSRSADAPAYQQGQNQLYNELNLGRREEYDVLDKRRGRDPEMGGKPRRKNPQEGLYNELQKDKMAEAYSEIGMKGERRRGKGHDGLYQGLSTATKDTYDALHMQALPPR

SEQ ID NO: 22 - protein, 452 aa, Artificial Sequence
  fusion P2A hFOXP3
GATNFSLLKQAGDVEENPGPSMPNPRPGKPSAPSLALGPSPGASPSWRAAPKASDLLGARGPGGTFQGRDLRGGAHASSSSLNPMPPSQLQLPTLPLVMVAPSGARLGPLPHLQALLQDRPHFMHQLSTVDAHARTPVLQVHPLESPAMISLTPPTTATGVFSLKARPGLPPGINVASLEWVSREPALLCTFPNPSAPRKDSTLSAVPQSSYPLLANGVCKWPGCEKVFEEPEDFLKHCQADHLLDEKGRAQCLLQREMVQSLEQQLVLEKEKLSAMQAHLAGKMALTKASSVASSDKGSCCIVAAGSQGPVVPAWSGPREAPDSLFAVRRHLWGSHGNSTFPEFLHNMDYFKFHNMRPPFTYATLIRWAILEAPEKQRTLNEIYHWFTRMFAFFRNHPATWKNAIRHNLSLHKCFVRVESEKGAVWTVDELEFRKKRSQRPSRCSNPTPGP

SEQ ID NO: 23 - protein, 280 aa, Artificial Sequence; identical to SEQ ID NO: 20
  ΔLNGFR (reporter)

SEQ ID NO: 24 - protein, 21 aa, Artificial Sequence
  secretory leader peptide
MALPVTALLLPLALLLHAAAP

SEQ ID NO: 25 - protein, 25 aa, Artificial Sequence
  secretory leader peptide
MDFQVQIFSFLLISASVIMSRGVHS